European Patent Application EP 4 775 677 A1, published July 15, 2026. Title: A microorganism of Corynebacterium genus having enhanced L-arginine productivity and a method for producing L-arginine using the same. Applicant: DAESANG CORPORATION. The sequence listing filed with the application follows.

SEQUENCE LISTING (14 sequences)

SEQ ID NO: 1 - protein, 211 aa, Escherichia coli
MFSYYFQGLALGAAMILPLGPQNAFVMNQGIRRQYHIMIALLCAISDLVLICAGIFGGSALLMQSPWLLALVTWGGVAFLLWYGFGAFKTAMSSNIELASAEVMKQGRWKIIATMLAVTWLNPHVYLDTFVVLGSLGGQLDVEPKRWFALGTISASFLWFFGLALLAAWLAPRLRTAKAQRIINLVVGCVMWFIALQLARDGIAHAQALFS

SEQ ID NO: 2 - DNA, 636 bp, Escherichia coli
  source 1..636: mol_type = genomic DNA
atgttctcctactacttccaaggcctggcgcttggtgcagccatgattttgcctttaggtccacaaaatgcctttgtgatgaaccagggtattcgacgtcagtaccacatcatgatcgctttgctgtgcgccatttctgatttggtgctgatctgtgcaggcatcttcggtggatctgccctgctcatgcagtccccgtggttgctcgctcttgtgacgtggggcggagtagcttttctgctgtggtatggtttcggcgcattcaaaaccgcgatgagctccaacatcgaactcgcatcagcagaagtcatgaagcagggccgctggaagattattgcaaccatgctggcagtgacctggcttaatccccatgtttatctcgacacttttgtcgtgcttgggtcgttgggtgggcagctcgatgttgagccaaagcgttggtttgcgctcggcaccatcagcgcttccttcctctggttcttcggacttgctttgctagctgcgtggctggcccctcgcctgaggacagcgaaagctcaacgcatcatcaacctggttgtcggctgcgtcatgtggttcatcgcactgcagcttgcacgcgacggcattgcccacgcccaagcgttgtttagttaa

SEQ ID NO: 3 - DNA, 32 bp, synthetic construct
  source 1..32: mol_type = other DNA
tgattacgcccggatccagatactcctttgga

SEQ ID NO: 4 - DNA, 22 bp, synthetic construct
  source 1..22: mol_type = other DNA
cggatccagatactcctttgga

SEQ ID NO: 5 - DNA, 20 bp, synthetic construct
  source 1..20: mol_type = other DNA
ttttggaatcggtggccttc

SEQ ID NO: 6 - DNA, 20 bp, synthetic construct
  source 1..20: mol_type = other DNA
ttttcgcgggttttggaatc

SEQ ID NO: 7 - DNA, 28 bp, synthetic construct
  source 1..28: mol_type = other DNA
cccgcgaaaatggcgggtattttcatcc

SEQ ID NO: 8 - DNA, 21 bp, synthetic construct
  source 1..21: mol_type = other DNA
tggcgggtattttcatccaaa

SEQ ID NO: 9 - DNA, 20 bp, synthetic construct
  source 1..20: mol_type = other DNA
tcctccaaaattgtggtggc

SEQ ID NO: 10 - DNA, 26 bp, synthetic construct
  source 1..26: mol_type = other DNA
gttcttgtaatcctccaaaattgtgg

SEQ ID NO: 11 - DNA, 34 bp, synthetic construct
  source 1..34: mol_type = other DNA
ttacaagaacatgttctcctactacttccaaggc

SEQ ID NO: 12 - DNA, 24 bp, synthetic construct
  source 1..24: mol_type = other DNA
atgttctcctactacttccaaggc

SEQ ID NO: 13 - DNA, 21 bp, synthetic construct
  source 1..21: mol_type = other DNA
attacccttccatcaccatcg

SEQ ID NO: 14 - DNA, 21 bp, synthetic construct
  source 1..21: mol_type = other DNA
gtcaccaacgattacccttcc